European Patent Application EP 4 393 951 A1, published July 3, 2024. Title: 抗Nectin-4抗体、药物缀合物及其制备方法和用途. Applicant: 石药集团巨石生物制药有限公司. Application CN. The sequence listing filed with the application follows.

SEQUENCE LISTING (17 sequences)

SEQ ID NO: 1 - protein, 8 aa, synthetic construct
GYTFTSYY

SEQ ID NO: 2 - protein, 8 aa, synthetic construct
IYPGNVNT

SEQ ID NO: 3 - protein, 9 aa, synthetic construct
ARGIYYFDY

SEQ ID NO: 4 - protein, 6 aa, synthetic construct
QSVNND

SEQ ID NO: 5 - skipped

SEQ ID NO: 6 - protein, 9 aa, synthetic construct
HQDYSSPFT

SEQ ID NO: 7 - protein, 116 aa, synthetic construct
QVQLQQSGPVLVKPGASVRISCKASGYTFTSYYIHWVKQRPGQGLEWIGWIYPGNVNTKYNENFRDKATLTADKSSSTSYMQLSSLTSEDSAVYFCARGIYYFDYWGQGTTLTVSS

SEQ ID NO: 8 - protein, 107 aa, synthetic construct
IIVMTQTPKFLLVSAGDRVTITCKASQSVNNDVAWYQEKPGQSPKLLIYYASNRDTGVPDRFTGSGYGTDFTFTISTVQAEDLAVYFCHQDYSSPFTFGSGTKLEIK

SEQ ID NO: 9 - protein, 116 aa, synthetic construct
QVQLVQSGAEVKKPGASVKVSCKASGYTFTSYYIHWVRQAPGQRLEWMGWIYPGNVNTKYNENFRDRVTITRDTSASTAYMELSSLRSEDTAVYYCARGIYYFDYWGQGTLVTVSS

SEQ ID NO: 10 - protein, 107 aa, synthetic construct
IIQMTQSPKFLSASVGDRVTITCKASQSVNNDVAWYQQKPGQSPKLLIYYASNRDTGVPDRFSGSGSGTDFTLTISSLQPEDFATYFCHQDYSSPFTFGGGTKVEIK

SEQ ID NO: 11 - protein, 107 aa, synthetic construct
AIQMTQSPSSLSASVGDRVTITCKASQSVNNDVAWYQQKPGKAPKLLIYYASNRDTGVPSRFSGSGSGTDFTLTISSLQAEDLAVYFCHQDYSSPFTFGGGTKVEIK

SEQ ID NO: 12 - protein, 107 aa, synthetic construct
AIQMTQSPSSLSASVGDRVTITCKASQSVNNDVAWYQQKPGKAPKLLIYYASNRDTGVPSRFSGSGSGTDFTLTISSLQPEDFATYFCHQDYSSPFTFGGGTKVEIK

SEQ ID NO: 13 - protein, 331 aa, synthetic construct
DSDERVTPPAEPLDRMPDPYRPSYGRAETIVNNYIRKWQQVYSHRDGRKQQMTEEQREWLSYGCVGVTWVNSGQYPTNRLAFAFFDEDKYKNELKNGRPRSGETRAEFEGRVAKDSFDEAKGFQRARDVASVMNKALENAHDEGAYLDNLKKELANGNDALRNEDARSPFYSALRNTPSFKDRNGGNHDPSKMKAVIYSKHFWSGQDRSGSSDKRKYGDPEAFRPDRGTGLVDMSRDRNIPRSPTSPGESFVNFDYGWFGAQTEADADKTVWTHGNHYHAPNGSLGAMHVYESKFRNWSDGYSDFDRGAYVVTFVPKSWNTAPDKVTQGWP

SEQ ID NO: 14 - protein, 19 aa, synthetic construct
MELGLCWVFLVAILEGVQC

SEQ ID NO: 15 - protein, 22 aa, synthetic construct
MDMRVPAQLLGLLLLWFPGSRC

SEQ ID NO: 16 - protein, 330 aa, synthetic construct
ASTKGPSVFPLAPSSKSTSGGTAALGCLVKDYFPEPVTVSWNSGALTSGVHTFPAVLQSSGLYSLSSVVTVPSSSLGTQTYICNVNHKPSNTKVDKKVEPKSCDKTHTCPPCPAPELLGGPSVFLFPPKPKDTLMISRTPEVTCVVVDVSHEDPEVKFNWYVDGVEVHNAKTKPREEQYNSTYRVVSVLTVLHQDWLNGKEYKCKVSNKALPAPIEKTISKAKGQPREPQVYTLPPSREEMTKNQVSLTCLVKGFYPSDIAVEWESNGQPENNYKTTPPVLDSDGSFFLYSKLTVDKSRWQQGNVFSCSVMHEALHNHYTQKSLSLSPGK

SEQ ID NO: 17 - protein, 107 aa, synthetic construct [sequence omitted]